European Patent Specification EP 3 686 214 B1, published July 1, 2026. Title: cAMP receptor protein variant and method for producing L-amino acid using the same. Applicant: CJ CheilJedang Corporation. The sequence listing filed with the application follows.

SEQUENCE LISTING (7 sequences)

SEQ ID NO: 1 - protein, 210 aa, Unknown
  CRP
MVLGKPQTDPTLEWFLSHCHIHKYPSKSKLIHQGEKAETLYYIVKGSVAVLIKDEEGKEMILSYLNQGDFIGELGLFEEGQERSAWVRAKTACEVAEISYKKFRQLIQVNPDILMRLSAQMARRLQVTSEKVGNLAFLDVTGRIAQTLLNLAKQPDAMTHPDGMQIKITRQEIGQIVGCSRETVGRILKMLEDQNLISAHGKTIVVYGTR

SEQ ID NO: 2 - DNA, 633 bp, Unknown
  crp
atggtgcttggcaaaccgcaaacagacccgactctcgaatggttcttgtctcattgccacattcataagtacccatccaagagcaagcttattcaccagggtgaaaaagcggaaacgctgtactacatcgttaaaggctctgtggcagtgctgatcaaagacgaagagggtaaagaaatgatcctctcctatctgaatcagggtgattttattggcgaactgggcctgtttgaagagggccaggaacgtagcgcatgggtacgtgcgaaaaccgcctgtgaagtggctgaaatttcgtacaaaaaatttcgccaattgattcaggtaaacccggacattctgatgcgtttgtctgcacagatggcgcgtcgtctgcaagtcacttcagagaaagtgggcaacctggcgttcctcgacgtgacgggccgcattgcacagactctgctgaatctggcaaaacaaccagacgctatgactcacccggacggtatgcaaatcaaaattacccgtcaggaaattggtcagattgtcggctgttctcgtgaaaccgtgggacgcattctgaagatgctggaagatcagaacctgatctccgcacacggtaaaaccatcgtcgtttacggcactcgttaa

SEQ ID NO: 3 - protein, 210 aa, Unknown
  modified CRP
MVLGKPQTDPTLEWFLSHCHIHKYPSKSKLIHKGEKAETLYYIVKGSVAVLIKDEEGKEMILSYLNQGDFIGELGLFEEGQERSAWVRAKTACEVAEISYKKFRQLIQVNPDILMRLSAQMARRLQVTSEKVGNLAFLDVTGRIAQTLLNLAKQPDAMTHPDGMQIKITRQEIGQIVGCSRETVGRILKMLEDQNLISAHGKTIVVYGTR

SEQ ID NO: 4 - DNA, 633 bp, Unknown
  modified crp
atggtgcttggcaaaccgcaaacagacccgactctcgaatggttcttgtctcattgccacattcataagtacccatccaagagcaagcttattcacaagggtgaaaaagcggaaacgctgtactacatcgttaaaggctctgtggcagtgctgatcaaagacgaagagggtaaagaaatgatcctctcctatctgaatcagggtgattttattggcgaactgggcctgtttgaagagggccaggaacgtagcgcatgggtacgtgcgaaaaccgcctgtgaagtggctgaaatttcgtacaaaaaatttcgccaattgattcaggtaaacccggacattctgatgcgtttgtctgcacagatggcgcgtcgtctgcaagtcacttcagagaaagtgggcaacctggcgttcctcgacgtgacgggccgcattgcacagactctgctgaatctggcaaaacaaccagacgctatgactcacccggacggtatgcaaatcaaaattacccgtcaggaaattggtcagattgtcggctgttctcgtgaaaccgtgggacgcattctgaagatgctggaagatcagaacctgatctccgcacacggtaaaaccatcgtcgtttacggcactcgttaa

SEQ ID NO: 5 - DNA, 933 bp, Unknown
  crp and expression control region
tttgctactccactgcgtcaattttcctgacagagtacgcgtactaaccaaatcgcgcaacggaaggcgacctgggtcatgctgaagcgagacaccaggagacacaaagcgaaagctatgctaaaacagtcaggatgctacagtaatacattgatgtactgcatgtatgcaaaggacgtcacattaccgtgcagtacagttgatagccccttcccaggtagcgggaagcatatttcggcaatccagagacagcggcgttatctggctctggagaaagcttataacagaggataaccgcgcatggtgcttggcaaaccgcaaacagacccgactctcgaatggttcttgtctcattgccacattcataagtacccatccaagagcaagcttattcaccagggtgaaaaagcggaaacgctgtactacatcgttaaaggctctgtggcagtgctgatcaaagacgaagagggtaaagaaatgatcctctcctatctgaatcagggtgattttattggcgaactgggcctgtttgaagagggccaggaacgtagcgcatgggtacgtgcgaaaaccgcctgtgaagtggctgaaatttcgtacaaaaaatttcgccaattgattcaggtaaacccggacattctgatgcgtttgtctgcacagatggcgcgtcgtctgcaagtcacttcagagaaagtgggcaacctggcgttcctcgacgtgacgggccgcattgcacagactctgctgaatctggcaaaacaaccagacgctatgactcacccggacggtatgcaaatcaaaattacccgtcaggaaattggtcagattgtcggctgttctcgtgaaaccgtgggacgcattctgaagatgctggaagatcagaacctgatctccgcacacggtaaaaccatcgtcgtttacggcactcgttaa

SEQ ID NO: 6 - DNA, 29 bp, Artificial Sequence
  crp-F
cacgaattctttgctactccactgcgtca

SEQ ID NO: 7 - DNA, 29 bp, Artificial Sequence
  crp-R
acacgaattcttaacgagtgccgtaaacg